European Patent Application EP 4 603 586 A1, published August 20, 2025. Title: Inhibitory oligonucleotides against ADAMTS7. Applicant: Universität zu Lübeck. Application EP. The sequence listing filed with the application follows.

SEQUENCE LISTING (39 sequences)

SEQ ID NO: 1 - RNA, 23 nt, Homo sapiens
  source 1..23: mol_type = mRNA
cagttttggcattcagcatgacg

SEQ ID NO: 2 - RNA, 23 nt, Homo sapiens
  source 1..23: mol_type = mRNA
cacagttttggcattcagcatga

SEQ ID NO: 3 - RNA, 23 nt, Homo sapiens
  source 1..23: mol_type = mRNA
catgtctccacagctcctgtacg

SEQ ID NO: 4 - RNA, 23 nt, Homo sapiens
  source 1..23: mol_type = mRNA
tccaacgaggactacttcattga

SEQ ID NO: 5 - RNA, 23 nt, Homo sapiens
  source 1..23: mol_type = mRNA
gcagaaaagcatcaacatgaagg

SEQ ID NO: 6 - RNA, 23 nt, Homo sapiens
  source 1..23: mol_type = mRNA
aagatgaggaggaggacctaaag

SEQ ID NO: 7 - RNA, 23 nt, Homo sapiens
  source 1..23: mol_type = mRNA
tgaggaggaggacctaaagatca

SEQ ID NO: 8 - RNA, 21 nt, synthetic construct
  source 1..21: mol_type = other RNA
tcatgctgaatgccaaaactg

SEQ ID NO: 9 - RNA, 21 nt, synthetic construct
  source 1..21: mol_type = other RNA
gttttggcattcagcatgacg

SEQ ID NO: 10 - RNA, 21 nt, synthetic construct
  source 1..21: mol_type = other RNA
atgctgaatgccaaaactgtg

SEQ ID NO: 11 - RNA, 21 nt, synthetic construct
  source 1..21: mol_type = other RNA
cagttttggcattcagcatga

SEQ ID NO: 12 - RNA, 21 nt, synthetic construct
  source 1..21: mol_type = other RNA
tacaggagctgtggagacatg

SEQ ID NO: 13 - RNA, 21 nt, synthetic construct
  source 1..21: mol_type = other RNA
tgtctccacagctcctgtacg

SEQ ID NO: 14 - RNA, 21 nt, synthetic construct
  source 1..21: mol_type = other RNA
aatgaagtagtcctcgttgga

SEQ ID NO: 15 - RNA, 21 nt, synthetic construct
  source 1..21: mol_type = other RNA
caacgaggactacttcattga

SEQ ID NO: 16 - RNA, 21 nt, synthetic construct
  source 1..21: mol_type = other RNA
ttcatgttgatgcttttctgc

SEQ ID NO: 17 - RNA, 21 nt, synthetic construct
  source 1..21: mol_type = other RNA
agaaaagcatcaacatgaagg

SEQ ID NO: 18 - RNA, 21 nt, synthetic construct
  source 1..21: mol_type = other RNA
ttaggtcctcctcctcatctt

SEQ ID NO: 19 - RNA, 21 nt, synthetic construct
  source 1..21: mol_type = other RNA
gatgaggaggaggacctaaag

SEQ ID NO: 20 - RNA, 21 nt, synthetic construct
  source 1..21: mol_type = other RNA
atctttaggtcctcctcctca

SEQ ID NO: 21 - RNA, 21 nt, synthetic construct
  source 1..21: mol_type = other RNA
aggaggaggacctaaagatca

SEQ ID NO: 22 - RNA, 23 nt, synthetic construct
  source 1..23: mol_type = other RNA
cgtcatgctgaatgccaaaactg

SEQ ID NO: 23 - RNA, 22 nt, synthetic construct
  source 1..22: mol_type = other RNA
tcatgctgaatgccaaaactgt

SEQ ID NO: 24 - RNA, 22 nt, synthetic construct
  source 1..22: mol_type = other RNA
gtacaggagctgtggagacatg

SEQ ID NO: 25 - RNA, 22 nt, synthetic construct
  source 1..22: mol_type = other RNA
caatgaagtagtcctcgttgga

SEQ ID NO: 26 - RNA, 22 nt, synthetic construct
  source 1..22: mol_type = other RNA
cttcatgttgatgcttttctgc

SEQ ID NO: 27 - RNA, 22 nt, synthetic construct
  source 1..22: mol_type = other RNA
tttaggtcctcctcctcatctt

SEQ ID NO: 28 - RNA, 22 nt, synthetic construct
  source 1..22: mol_type = other RNA
gatctttaggtcctcctcctca

SEQ ID NO: 29 - DNA, 19 bp, synthetic construct
  source 1..19: mol_type = other DNA
atgctgaatgccaaaactg

SEQ ID NO: 30 - DNA, 21 bp, synthetic construct
  source 1..21: mol_type = other DNA
atgctgaatgccaaaactgtg

SEQ ID NO: 31 - DNA, 21 bp, synthetic construct
  source 1..21: mol_type = other DNA
tacaggagctgtggagacatg

SEQ ID NO: 32 - DNA, 21 bp, synthetic construct
  source 1..21: mol_type = other DNA
aatgaagtagtcctcgttgga

SEQ ID NO: 33 - DNA, 21 bp, synthetic construct
  source 1..21: mol_type = other DNA
ttcatgttgatgcttttctgc

SEQ ID NO: 34 - DNA, 20 bp, synthetic construct
  source 1..20: mol_type = other DNA
atggtgcgtgatctttaggt

SEQ ID NO: 35 - DNA, 20 bp, synthetic construct
  source 1..20: mol_type = other DNA
atggtgcgtgatctttaggt

SEQ ID NO: 36 - RNA, 18 nt, synthetic construct
  source 1..18: mol_type = other RNA
gcacctgtggagtgcaag

SEQ ID NO: 37 - RNA, 19 nt, synthetic construct
  source 1..19: mol_type = other RNA
gcgggtagccagacggtaa

SEQ ID NO: 38 - RNA, 19 nt, synthetic construct
  source 1..19: mol_type = other RNA
gcagcgatcagtcagcaaa

SEQ ID NO: 39 - RNA, 21 nt, synthetic construct
  source 1..21: mol_type = other RNA
agaagagcaccaatatgcagg